European Patent Application EP 4 711 453 A1, published March 18, 2026. Title: 苯丙氨酸裂解酶突变体及其偶联物或其药学上可接受的盐. Applicant: 重庆派金生物科技有限公司. Application CN. The sequence listing filed with the application follows.

SEQUENCE LISTING (11 sequences)

SEQ ID NO: 1 - protein, 567 aa, synthetic construct
MKTLSQAQSKTSSQQFSFTGNSSANVIIGNQKLTINDVARVARNGTLVSLTNNTDILQGIQASCDYINNAVESGEPIYGVTSGFGGMANVAISREQASELQTNLVWFLKTGAGNKLPLADVRAAMLLRANSHMRGASGIRLELIKRMEIFLNAGVTPYVYEFGSIGASGDLVPLSYITGSLIGLDPSFKVDFNGKEMDAPTALRQLNLSPLTLLPKEGLAMMNGTSVMTGIAANCVYDTQILTAIAMGVHALDIQALNGTNQSFHPFIHNSKPHPGQLWAADQMISLLANSQLVRDELDGKHDYRDHELIQDRYSLRCLPQYLGPIVDGISQIAKQIEIEINSVTDNPLIDVDNQASYHGGNFLGQYVGMGMDHLRYYIGLLAKHLDVQIALLASPEFSNGLPPSLLGNRERKVNMGLKGLQICGNSIMPLLTFYGNSIADRFPTHAEQFNQNINSQGYTSATLARRSVDIFQNYVAIALMFGVQAVDLRTYKKTGHYDARASLSPATERLYSAVRHVVGQKPTSDRPYIWNDNEQGLDEHIARISADIAAGGVIVQAVQDILPSLH

SEQ ID NO: 2 - protein, 567 aa, synthetic construct
MKTLSQAQSKTSSQQFSFTGNSSANVIIGNQKLTINDVARVARNGTLVSLTNNTDILQGIQASCDYINNAVESGEPIYGVTSGFGGMANVAISREQASELQTNLVWFLKTGAGNKLPLADVRAAMLLRANSHMRGASGIRLELIKRMEIFLNAGVTPYVYEFGSIGASGDLVPLSYITGSLIGLDPSFKVDFNGKEMDAPTALRQLNLSPLTLLPKEGLAMMNGTSVMTGIAANCVYDTQILTAIAMGVHALDIQALNGTNQSFHPFIHNSKPHPGQLWAADQMISLLANSQLVRDELDGKHDYRDHELIQDRYSLRCLPQYLGPIVDGISQIAKQIEIEINSVTDNPLIDVDNQASYHGGNFLGQYVGMGMDHLRYYIGLLAKHLDVQIALLASPEFSNGLPPSLLGNRERKVNMGLKGLQICGNSIMPLLTFYGNSIADRFPTHAEQFNQNINSQGYTSATLARRSVDIFQNYVAIALMFGVQAVDLRTYKKTGHYDARACLSPATERLYSAVRHVVGQKPTSDRPYIWNDNEQGLDEHIARISADIAAGGVIVQAVQDILPCLH

SEQ ID NO: 3 - protein, 569 aa, synthetic construct
MNITSLQQNITRSWQIPFTNSSDSIVTVGDRNLTIDEVVNVARHGTQVRLTDNADVIRGVQASCDYINNAVETAQPIYGVTSGFGGMADVVISREQAAELQTNLIWFLKSGAGNKLSLADVRAAMLLRANSHLYGASGIRLELIQRIETFLNAGVTPHVYEFGSIGASGDLVPLSYITGALIGLDPSFTVDFDGKEMDAVTALSRLGLPKLQLQPKEGLAMMNGTSVMTGIAANCVYDAKVLLALTMGVHALAIQGLYGTNQSFHPFIHQCKPHPGQLWTADQMFSLLKDSSLVREELDGKHEYRGKDLIQDRYSLRCLAQFIGPIVDGVSEITKQIEVEMNSVTDNPLIDVENQVSYHGGNFLGQYVGVTMDRLRYYIGLLAKHIDVQIALLVSPEFSNGLPPSLVGNSDRKVNMGLKGLQISGNSIMPLLSFYGNSLADRFPTHAEQFNQNINSQGYISANLTRRSVDIFQNYMAIALMFGVQAVDLRTYKMKGHYDARTCLSPNTVQLYTAVCEVVGKPLTSVRPYIWNDNEQCLDEHIARISADIAGGGLIVQAVEHIFSSLKST

SEQ ID NO: 4 - protein, 567 aa, synthetic construct
MKTLSQAQSKTSSQQFSFTGNSSANVIIGNQKLTINDVARVARNGTLVSLTNNTDILQGIQASCDYINNAVESGEPIYGVTSGFGGMANVAISREQASELQTNLVWFLKTGAGNKLPLADVRAAMLLRANSHMRGASGIRLELIKRMEIFLNAGVTPYVYEFGSIGASGDLVPLSYITGSLIGLDPSFKVDFNGKEMDAPTALRQLNLSPLTLLPKEGLAMMNGTSVMTGIAANCVYDTQILTAIAMGVHALDIQALNGTNQSFHPFIHNSKPHPGQLWAADQMISLLANSQLVRDELDGKHDYRDHELIQDRYSLRCLPQYLGPIVDGISQIAKQIEIEINSVTDNPLIDVDNQASYHGGNFLGQYVGMGMDHLRYYIGLLAKHLDVQIALLASPEFSNGLPPSLLGNRERKVNMGLKGLQICGNSIMPLLTFYGNSIADRFPTHAEQFNQNINSQGYTSATLARKSVDIFQNYVAIALMFGVQAVDLRTYKKTGHYDARASLSPATERLYSAVRHVVGQKPTSDRPYIWNDNEQGLDEHIAKISADIAAGGVIVQAVQDILPSLH

SEQ ID NO: 5 - protein, 567 aa, synthetic construct
MKTLSQAQSKTSSQQFSFTGNSSANVIIGNQKLTINDVARVARNGTLVSLTNNTDILQGIQASCDYINNAVKSGEPIYGVTSGFGGMANVAISREQASELQTNLVWFLKTGAGNKLPLADVRAAMLLRANSHMRGASGIRLELIKRMEIFLNAGVTPYVYEFGSIGASGDLVPLSYITGSLIGLDPSFKVDFNGKEMDAPTALRQLNLSPLTLLPKEGLAMMNGTSVMTGIAANCVYDTQILTAIAMGVHALDIQALNGTNQSFHPFIHNSKPHPGQLWAADQMISLLANSQLVRDELDGKHDYRDHELIQDRYSLRCLPQYLGPIVDGISQIAKQIEIEINSVTDNPLIDVDNQASYHGGNFLGQYVGMGMDHLRYYIGLLAKHLDVQIALLASPEFSNGLPPSLLGNRERKVNMGLKGLQICGNSIMPLLTFYGNSIADRFPTHAEQFNQNINSQGYTSATLARKSVDIFQNYVAIALMFGVQAVDLRTYKKTGHYDARASLSPATERLYSAVRHVVGQKPTSDRPYIWNDNEQGLDEHIAKISADIAAGGVIVQAVQDILPSLH

SEQ ID NO: 6 - protein, 567 aa, synthetic construct
MKTLSQAQSKTSSQQFSFTGNSSANVIIGNQKLTINDVARVARNGTLVSLTNNTDILQGIQASCDYINNAVKSGEPIYGVTSGFGGMANVAISREQASELQTNLVWFLKTGAGNKLPLADVRAAMLLRANSHMRGASGIRLELIKRMEIFLNAGVTPYVYEFGSIGASGDLVPLSYITGSLIGLDPSFKVDFNGKEMDAPTALRQLNLSPLTLLPKEGLAMMNGTSVMTGIAANCVYDTKILTAIAMGVHALDIQALNGTNQSFHPFIHNSKPHPGQLWAADQMISLLANSQLVRDELDGKHDYRDHELIQDRYSLRCLPQYLGPIVDGISQIAKQIEIEINSVTDNPLIDVDNQASYHGGNFLGQYVGMGMDHLRYYIGLLAKHLDVQIALLASPEFSNGLPPSLLGNRERKVNMGLKGLQICGNSIMPLLTFYGNSIADRFPTHAEQFNQNINSQGYTSATLARKSVDIFQNYVAIALMFGVQAVDLRTYKKTGHYDARASLSPATERLYSAVRHVVGQKPTSDRPYIWNDNEQGLDEHIAKISADIAAGGVIVQAVQDILPSLH

SEQ ID NO: 7 - protein, 566 aa, synthetic construct
MKTLSQAQSKTSSQQFSFTGNSSANVIIGNQKLTINDVARVARNGTLVSLTNNTDILQGIQASCDYINNAVESGEPIYGVTSGFGGMANVAISREQASELQTNLVWFLKTGAGNKLPLADVRAAMLLRANSHMRGASGIRLELIKRMEIFLNAGVTPYVYEFGSIGASGDLVPLSYITGSLIGLDPSFKVDFNGKEMDAPTALRQLNLSPLTLLPKEGLAMMNGTSVMTGIAANCVYDTQILTAIAMGVHALDIQALNGTNQSFHPFIHNSKPHPGQLWAADQMISLLANSQLVRDELDGKHDYRDHELIQDRYSLRCLPQYLGPIVDGISQIAKQIEIEINSVTDNPLIDVDNQASYHGGNFLGQYVGMGMDHLRYYIGLLAKHLDVQIALLASPEFSNGLPPSLLGNRERKVNMGLKGLQICGNSIMPLLTFYGNSIADRFPTHAEQFNQNINSQGYTSATLARKSVDIFQNYVAIALMFGVQAVDLRTYKKTGHYDARACLSPATERLYSAVRHVVGQKPTSDRPYIWNDNEQGLDEHIAKISAIAAGGVIVQAVQDILPCLH

SEQ ID NO: 8 - protein, 566 aa, synthetic construct
MKTLSQAQSKTSSQQFSFTGNSSANVIIGNQKLTINDVARVARNGTLVSLTNNTDILQGIQASCDYINNAVKSGEPIYGVTSGFGGMANVAISREQASELQTNLVWFLKTGAGNKLPLADVRAAMLLRANSHMRGASGIRLELIKRMEIFLNAGVTPYVYEFGSIGASGDLVPLSYITGSLIGLDPSFKVDFNGKEMDAPTALRQLNLSPLTLLPKEGLAMMNGTSVMTGIAANCVYDTQILTAIAMGVHALDIQALNGTNQSFHPFIHNSKPHPGQLWAADQMISLLANSQLVRDELDGKHDYRDHELIQDRYSLRCLPQYLGPIVDGISQIAKQIEIEINSVTDNPLIDVDNQASYHGGNFLGQYVGMGMDHLRYYIGLLAKHLDVQIALLASPEFSNGLPPSLLGNRERKVNMGLKGLQICGNSIMPLLTFYGNSIADRFPTHAEQFNQNINSQGYTSATLARKSVDIFQNYVAIALMFGVQAVDLRTYKKTGHYDARACLSPATERLYSAVRHVVGQKPTSDRPYIWNDNEQGLDEHIAKISAIAAGGVIVQAVQDILPCLH

SEQ ID NO: 9 - protein, 566 aa, synthetic construct
MKTLSQAQSKTSSQQFSFTGNSSANVIIGNQKLTINDVARVARNGTLVSLTNNTDILQGIQASCDYINNAVKSGEPIYGVTSGFGGMANVAISREQASELQTNLVWFLKTGAGNKLPLADVRAAMLLRANSHMRGASGIRLELIKRMEIFLNAGVTPYVYEFGSIGASGDLVPLSYITGSLIGLDPSFKVDFNGKEMDAPTALRQLNLSPLTLLPKEGLAMMNGTSVMTGIAANCVYDTKILTAIAMGVHALDIQALNGTNQSFHPFIHNSKPHPGQLWAADQMISLLANSQLVRDELDGKHDYRDHELIQDRYSLRCLPQYLGPIVDGISQIAKQIEIEINSVTDNPLIDVDNQASYHGGNFLGQYVGMGMDHLRYYIGLLAKHLDVQIALLASPEFSNGLPPSLLGNRERKVNMGLKGLQICGNSIMPLLTFYGNSIADRFPTHAEQFNQNINSQGYTSATLARKSVDIFQNYVAIALMFGVQAVDLRTYKKTGHYDARACLSPATERLYSAVRHVVGQKPTSDRPYIWNDNEQGLDEHIAKISAIAAGGVIVQAVQDILPCLH

SEQ ID NO: 10 - protein, 569 aa, synthetic construct
MNITSLQQNITRSWQIPFTNSSDSIVTVGDRNLTIDEVVNVARHGTQVRLTDNADVIRGVQASCDYINNAVETAQPIYGVTSGFGGMADVVISREQAAELQTNLIWFLKSGAGNKLSLADVRAAMLLRANSHLYGASGIRLELIQRIETFLNAGVTPHVYEFGSIGASGDLVPLSYITGALIGLDPSFTVDFDGKEMDAVTALSRLGLPKLQLQPKEGLAMMNGTSVMTGIAANCVYDAKVLLALTMGVHALAIQGLYGTNQSFHPFIHQCKPHPGQLWTADQMFSLLKDSSLVREELDGKHEYRGKDLIQDRYSLRCLAQFIGPIVDGVSEITKQIEVEMNSVTDNPLIDVENQVSYHGGNFLGQYVGVTMDRLRYYIGLLAKHIDVQIALLVSPEFSNGLPPSLVGNSDRKVNMGLKGLQISGNSIMPLLSFYGNSLADRFPTHAEQFNQNINSQGYISANLTRKSVDIFQNYMAIALMFGVQAVDLRTYKMKGHYDARTCLSPNTVQLYTAVCEVVGKPLTSVRPYIWNDNEQCLDEHIAKISADIAGGGLIVQAVEHIFSSLKST

SEQ ID NO: 11 - protein, 569 aa, synthetic construct
MNITSLQQNITRSWQIPFTNSSDSIVTVGDRNLTIDEVVNVARHGTQVRLTDNADVIRGVQASCDYINNAVKTAQPIYGVTSGFGGMADVVISREQAAELQTNLIWFLKSGAGNKLSLADVRAAMLLRANSHLYGASGIRLELIQRIETFLNAGVTPHVYEFGSIGASGDLVPLSYITGALIGLDPSFTVDFDGKEMDAVTALSRLGLPKLQLQPKEGLAMMNGTSVMTGIAANCVYDAKVLLALTMGVHALAIQGLYGTNQSFHPFIHQCKPHPGQLWTADQMFSLLKDSSLVREELDGKHEYRGKDLIQDRYSLRCLAQFIGPIVDGVSEITKQIEVEMNSVTDNPLIDVENQVSYHGGNFLGQYVGVTMDRLRYYIGLLAKHIDVQIALLVSPEFSNGLPPSLVGNSDRKVNMGLKGLQISGNSIMPLLSFYGNSLADRFPTHAEQFNQNINSQGYISANLTRKSVDIFQNYMAIALMFGVQAVDLRTYKMKGHYDARTCLSPNTVQLYTAVCEVVGKPLTSVRPYIWNDNEQCLDEHIAKISADIAGGGLIVQAVEHIFSSLKST